European Patent Application EP 4 349 351 A1, published April 10, 2024. Title: Extracellular Vesicles Derived from Lactobacillus plantarum and use thereof. Applicant: MD Healthcare Inc. The sequence listing filed with the application follows.

SEQUENCE LISTING (14 sequences)

SEQ ID NO: 1 - DNA, 20 bp, Artificial Sequence
  total Bdnf_F
tggctgacacttttgagcac

SEQ ID NO: 2 - DNA, 20 bp, Artificial Sequence
  total Bdnf_R
gtttgcggcatccaggtaat

SEQ ID NO: 3 - DNA, 20 bp, Artificial Sequence
  Bdnf1_F
cctgcatctgttggggagac

SEQ ID NO: 4 - DNA, 20 bp, Artificial Sequence
  Bdnf1_R
gccttgtccgtggacgttta

SEQ ID NO: 5 - DNA, 21 bp, Artificial Sequence
  Bdnf4_F
cagagcagctgccttgatgtt

SEQ ID NO: 6 - DNA, 20 bp, Artificial Sequence
  Bdnf4_R
gccttgtccgtggacgttta

SEQ ID NO: 7 - DNA, 18 bp, Artificial Sequence
  Ngf_F
agcattcccttgacacag

SEQ ID NO: 8 - DNA, 18 bp, Artificial Sequence
  Ngf_R
ggtctacagtgatgttgc

SEQ ID NO: 9 - DNA, 21 bp, Artificial Sequence
  Sirt1_F
gatccttcagtgtcatggttc

SEQ ID NO: 10 - DNA, 18 bp, Artificial Sequence
  Sirt1_R
atggcaagtggctcatca

SEQ ID NO: 11 - DNA, 20 bp, Artificial Sequence
  Hdac2_F
gggacaggcttggttgtttc

SEQ ID NO: 12 - DNA, 20 bp, Artificial Sequence
  Hdac2_R
gagcatcagcaatggcaagt

SEQ ID NO: 13 - DNA, 20 bp, Artificial Sequence
  Creb1_F
gaggcagcaagagaatgtcg

SEQ ID NO: 14 - DNA, 20 bp, Artificial Sequence
  Creb1_R
ccagtccattctccaccgta